European Patent Application EP 4 786 493 A1, published August 5, 2026. Title: 结合Claudin 18.2的结合部分及其应用. Applicant: 南京蓬勃生物科技有限公司. The sequence listing filed with the application follows.

SEQUENCE LISTING (47 sequences)

SEQ ID NO: 1 - protein, 118 aa, synthetic construct
QLQQVESGGGLVQPGGSLRLSCAASRNIGILSTMGWYRQAPGKQRELVATITRGGSTNYGEFVKGRFTISRDNAKNTVYLQMNSLKPEDTAVYYCNVDESWLGTQSYWGRGTTVTVSS

SEQ ID NO: 2 - protein, 8 aa, synthetic construct
RNIGILST

SEQ ID NO: 3 - protein, 7 aa, synthetic construct
ITRGGST

SEQ ID NO: 4 - protein, 12 aa, synthetic construct
NVDESWLGTQSY

SEQ ID NO: 5 - protein, 109 aa, synthetic construct
QSVLTQPASVSGSPGQSITISCTGTSSDVGGYKYVSWYQQPPGKAPKLIIYEVTKRPSGVPDRFSGSKSGNTASLTVSGLQAEDEADYYCLSYAGSNNVFGTGTKLTVL

SEQ ID NO: 6 - protein, 9 aa, synthetic construct
SSDVGGYKY

SEQ ID NO: 7 - skipped

SEQ ID NO: 8 - protein, 9 aa, synthetic construct
LSYAGSNNV

SEQ ID NO: 9 - protein, 121 aa, synthetic construct
QVQLQQSGGGSVQAGGSLRLSCAASGTILSINAMGWYRQAPGKQRELVATITTGGNANYAHSVKGRFTISRDNAKNTVYLQMNNLKPEDTAVYYCNAEQVVVGFLQAYDVWGQGTTVTVSS

SEQ ID NO: 10 - protein, 8 aa, synthetic construct
GTILSINA

SEQ ID NO: 11 - protein, 7 aa, synthetic construct
ITTGGNA

SEQ ID NO: 12 - protein, 15 aa, synthetic construct
NAEQVVVGFLQAYDV

SEQ ID NO: 13 - protein, 112 aa, synthetic construct
DVVMTQSPLSLPVTLGQAASISCRSSQSLVHGDGNTYLNWIQQRPGQSPRRLIYKVSNRDSGVPDRFSGSGSGTDFTLKISRVEAEDVGVYYCMQGTHWPSTFGPGTKVDIK

SEQ ID NO: 14 - protein, 11 aa, synthetic construct
QSLVHGDGNTY

SEQ ID NO: 15 - skipped

SEQ ID NO: 16 - protein, 9 aa, synthetic construct
MQGTHWPST

SEQ ID NO: 17 - protein, 118 aa, synthetic construct
QVQLMQSGGGLVQPGGSLRLSCAASRNIGILSTMGWYRQAPGKQRELVATITRGGSTNYGEFVKGRFTISRDNAKNTVYLQMNSLKPEDTAVYYCNVDESWLGTQSYWGRGTTVTVSS

SEQ ID NO: 18 - protein, 106 aa, synthetic construct
QSALTQPPSASGSPGQSVTISCTGTSSDIGTYNFVSWYQQHPGKAPKLIIYEVSKRPSGVPDRFSGSKSGNTASLTVSGLQAEDEADYYCKSYPRVFGTGTKLTAL

SEQ ID NO: 19 - protein, 9 aa, synthetic construct
SSDIGTYNF

SEQ ID NO: 20 - skipped

SEQ ID NO: 21 - protein, 6 aa, synthetic construct
KSYPRV

SEQ ID NO: 22 - protein, 118 aa, synthetic construct
QVQLMQSGGGLVQPGGSLRLSCAASRNIGILSTMGWYRQAPGKQRELVATITRGGSTNYGEFVKGRFTISRDNAKNTVYLQMNSLKPEDTAVYYCNVDESWLGTQSYWGRGTQVTVSS

SEQ ID NO: 23 - protein, 109 aa, synthetic construct
QAVVTQEPSLTVSPGGTVTLTCGSSTGPVTSGHYPHWYQQKPGQAPKTLIFDTSHKHPWTPAQFSGSLLGGKAALTLSGAHPEDEAEYYCLLSYSGVRVFGGGTQLIIL

SEQ ID NO: 24 - protein, 9 aa, synthetic construct
TGPVTSGHY

SEQ ID NO: 25 - skipped

SEQ ID NO: 26 - protein, 9 aa, synthetic construct
LLSYSGVRV

SEQ ID NO: 27 - protein, 118 aa, synthetic construct
QVQLQESGGGVVQPGGSLRLSCAASQSIGLLSTMGWYRQAAGKQRELVATITRGGSTNYGEFVKGRFTISRDNAKNTVYLQMNSLKPEDTAVYYCTADESWLGTQSYWGRGTRVTVSS

SEQ ID NO: 28 - protein, 8 aa, synthetic construct
QSIGLLST

SEQ ID NO: 29 - protein, 12 aa, synthetic construct
TADESWLGTQSY

SEQ ID NO: 30 - protein, 110 aa, synthetic construct
QAGLTQPPSASGTPGQGVTISCSGSSSNIGSNSVNWYQQLPGTAPKLLMHSNNERSSGVPDRFSGSKSGSSASLAISGLQSEDAADYFCGAWDDSLNGYVFGTGTKLTVL

SEQ ID NO: 31 - protein, 8 aa, synthetic construct
SSNIGSNS

SEQ ID NO: 32 - skipped

SEQ ID NO: 33 - protein, 11 aa, synthetic construct
GAWDDSLNGYV

SEQ ID NO: 34 - protein, 118 aa, synthetic construct
QVQLVQSGGGLVQPGGSLRLSCAASRNIGILSTMGWYRQAPGKQRELVATITRGGSTNYGEFVKGRFTISRDNAKNTVYLQMNSLKPEDTAVYYCNVDESWLGTQSYWGRGPLVTVSS

SEQ ID NO: 35 - protein, 107 aa, synthetic construct
DIVMTQSPSSVSASVGDRVTITCRASQGISSWLAWYQQKPGKAPKLLIYAASSLQSGVPSRFSGSGSGTDFTLTISSLQPEDFATYYCQQANSFPLTFGGGTKVEIK

SEQ ID NO: 36 - protein, 6 aa, synthetic construct
QGISSW

SEQ ID NO: 37 - skipped

SEQ ID NO: 38 - protein, 9 aa, synthetic construct
QQANSFPLT

SEQ ID NO: 39 - protein, 108 aa, synthetic construct
EIVMTQSPATLSVSPGERATLSCRASQSVSSNLAWYQQKPGQAPRLLIYGASTRATGIPARFSGSGSGTEFTLTISSLQSEDFAVYYCQQYNNWPPWTFGQGTKVEIK

SEQ ID NO: 40 - protein, 6 aa, synthetic construct
QSVSSN

SEQ ID NO: 41 - skipped

SEQ ID NO: 42 - protein, 10 aa, synthetic construct [sequence omitted]

SEQ ID NO: 43 - protein, 118 aa, synthetic construct
QVQLVDSGGGLVQSGGSLRLTCAASQSIGLLSTMGWYRQAAGKQRELVATITRGGSTNYGEFVKGRFTISRDNAKNTVYLQMNSLKPEDTAVYYCTADESWLGTQSYWGRGTLVTVSS

SEQ ID NO: 44 - protein, 113 aa, synthetic construct
DIVMTQSPDSLAVSLGERATINCKSSQSVLYSSNNKNYLAWYQQKPGQPPKLLIYWASTRESGVPDRFSGSGSGTDFTLTISSLQAEDVAVYYCQQYYSTPRTFGQGTKVEIK

SEQ ID NO: 45 - protein, 12 aa, synthetic construct
QSVLYSSNNKNY

SEQ ID NO: 46 - skipped

SEQ ID NO: 47 - protein, 9 aa, synthetic construct
QQYYSTPRT